European Patent Specification EP 3 221 449 B1, published August 30, 2023. Title: PROCESS FOR REFOLDING RECOMBINANT CHYMOTRYPSIN. Applicant: Sleevi, Mark C Lile, Jack Grimison, Bryn. The sequence listing filed with the application follows.

SEQUENCE LISTING (4 sequences)

SEQ ID NO: 1 - protein, 245 aa, Sus scrufa
CGVPAIPPVLSGLSRIVNGENAVPGSWPWQVSLQDGTGFHFCGGSLISEDWVVTAAHCGVTTSDVVVAGEYDQASDAEDIQVLKIAKVFKNPNFSLLTVRNDITLLKLATPARFSRTVSAVCLPSASDDFPAGTLCATTGWGKTKYTALKTPDKLQQAALPIVSSTVCKSYWGSKVTDVMICAGASGVSSCMGDSGGPLVCQKNGAWTLVGIVSWGSSTCSTTTPAVYARVTALIPWVQQILANN

SEQ ID NO: 2 - protein, 230 aa, Sus scrufa
IVNGENAVPGSWPWQVSLQDGTGFHFCGGSLISEDWVVTAAHCGVTTSDVVVAGEYDQASDAEDIQVLKIAKVFKNPNFSLLTVRNDITLLKLATPARFSRTVSAVCLPSASDDFPAGTLCATTGWGKTKYTALKTPDKLQQAALPIVSSTVCKSYWGSKVTDVMICAGASGVSSCMGDSGGPLVCQKNGAWTLVGIVSWGSSTCSTTTPAVYARVTALIPWVQQILANN

SEQ ID NO: 3 - protein, 254 aa, Artificial sequence
  modified chymotrypsin B with a leader of 6-8 amino acids
  VARIANT (2)..(2): X is any amino acid
  VARIANT (3)..(3): X is any amino acid
  VARIANT (4)..(4): X is any amino acid
  VARIANT (5)..(5): X is any amino acid
  VARIANT (6)..(6): X is any amino acid or absent
  VARIANT (7)..(7): X is any amino acid or absent
  VARIANT (8)..(8): X is F, W, or Y
  misc_feature (9)..(9): Xaa can be any naturally occurring amino acid
MXXXXXXXXCGVPAIPPVLSGLSRIVNGENAVPGSWPWQVSLQDGTGFHFCGGSLISEDWVVTAAHCGVTTSDVVVAGEYDQASDAEDIQVLKIAKVFKNPNFSLLTVRNDITLLKLATPARFSRTVSAVCLPSASDDFPAGTLCATTGWGKTKYTALKTPDKLQQAALPIVSSTVCKSYWGSKVTDVMICAGASGVSSCMGDSGGPLVCQKNGAWTLVGIVSWGSSTCSTTTPAVYARVTALIPWVQQILANN

SEQ ID NO: 4 - protein, 254 aa, Artificial sequence
  Chymotrypsin B with a 7 amino acid leader
  VARIANT (2)..(2): X is any amino acid or absent
  VARIANT (3)..(3): X is any amino acid
  VARIANT (4)..(4): X is any amino acid
  VARIANT (5)..(5): X is any amino acid
  VARIANT (6)..(6): X is any amino acid
  VARIANT (7)..(7): X is any amino acid or absent
  misc_feature (8)..(8): Xaa can be any naturally occurring amino acid
MXXXXXXXFCGVPAIPPVLSGLSRIVNGENAVPGSWPWQVSLQDGTGFHFCGGSLISEDWVVTAAHCGVTTSDVVVAGEYDQASDAEDIQVLKIAKVFKNPNFSLLTVRNDITLLKLATPARFSRTVSAVCLPSASDDFPAGTLCATTGWGKTKYTALKTPDKLQQAALPIVSSTVCKSYWGSKVTDVMICAGASGVSSCMGDSGGPLVCQKNGAWTLVGIVSWGSSTCSTTTPAVYARVTALIPWVQQILANN